European Patent Application EP 4 563 149 A1, published June 4, 2025. Title: Compounds for use in the treatment of skin cancers. Applicant: PHARMA MAR, S.A. Application EP. The sequence listing filed with the application follows.

SEQUENCE LISTING (16 sequences)

SEQ ID NO: 1 - DNA, 25 bp, synthetic construct
  source 1..25: mol_type = other DNA
cattgttatgctggaaatgctagaa

SEQ ID NO: 2 - DNA, 23 bp, synthetic construct
  source 1..23: mol_type = other DNA
ggcttgctgtatgtggtacttgg

SEQ ID NO: 3 - DNA, 19 bp, synthetic construct
  source 1..19: mol_type = other DNA
ccgtggacctactctggct

SEQ ID NO: 4 - DNA, 19 bp, synthetic construct
  source 1..19: mol_type = other DNA
ccttggcgttatgggcttc

SEQ ID NO: 5 - DNA, 20 bp, synthetic construct
  source 1..20: mol_type = other DNA
acatctgctggaaggtggac

SEQ ID NO: 6 - DNA, 20 bp, synthetic construct
  source 1..20: mol_type = other DNA
cccagcacaatgaagatcaa

SEQ ID NO: 7 - DNA, 25 bp, synthetic construct
  source 1..25: mol_type = other DNA
ttgaggacctctgtgtatttgtcaa

SEQ ID NO: 8 - DNA, 23 bp, synthetic construct
  source 1..23: mol_type = other DNA
cctggaggagaagaggaaagaga

SEQ ID NO: 9 - DNA, 20 bp, synthetic construct
  source 1..20: mol_type = other DNA
cggctgtttaacttcgcttc

SEQ ID NO: 10 - DNA, 20 bp, synthetic construct
  source 1..20: mol_type = other DNA
cacacgccaagaaacagtga

SEQ ID NO: 11 - DNA, 25 bp, synthetic construct
  source 1..25: mol_type = other DNA
ccagtttgactactctgaccatcag

SEQ ID NO: 12 - DNA, 24 bp, synthetic construct
  source 1..24: mol_type = other DNA
atataggagaaggccgagtagagg

SEQ ID NO: 13 - DNA, 17 bp, synthetic construct
  source 1..17: mol_type = other DNA
gcagcgatgcgaccctc

SEQ ID NO: 14 - DNA, 21 bp, synthetic construct
  source 1..21: mol_type = other DNA
ccaactgcgtgagcttgttac

SEQ ID NO: 15 - DNA, 24 bp, synthetic construct
  source 1..24: mol_type = other DNA
tcaactttcgatggtagtcgccgt

SEQ ID NO: 16 - DNA, 24 bp, synthetic construct
  source 1..24: mol_type = other DNA
tccttggatgtggtagccgtttct